European Patent Specification EP 3 488 003 B1, published October 25, 2023. Title: NUCLEIC ACID CONTROL MOLECULES FROM NON-HUMAN ORGANISMS. Applicant: EXACT SCIENCES CORPORATION. The sequence listing filed with the application follows.

SEQUENCE LISTING (24 sequences)

SEQ ID NO: 1 - DNA, 2241 bp, Danio rerio
tcagcaaatgaagtctgctctccgttcgctcctcaaagtaggacagatcgcgccggattaagcgttaatctgagtcttctgcgcatgcgcatgaacgcgcgctacaagcggacaaggtgcgcgttcgaagaagaaacgaaccgagccggtttcgagcagcgacaacgcgaatgaagcccacggagtaccgaaaccttgaggaattcatctttctgccagcggaggactgttttcagtttagttttgagcgtaatggaagatgtttgggcacttttgcgcaatccctcatgttatcgcctcacagacacgcgtcgcgcgcgcagattacgcttaatttgagcggatttgaggaaacagacgcgtttactgtcagtcgaggctctactgaagactgaaagtggcttgtttgggtttaagattgacccagatgctactgaaaactgtcaatcaagaaggaaactcttgaagcaataaaaacatcatctctgttatatgaagactgtcagatccacacagtgatccatgtttgtggatatgcaaacacatcagaacgagacgctaaatttatcagcttgctttggagtaaacagcgttgctttaaaacactccacagtcataaatcatctccagccctaaccatggtccactgagccatgccgttcatcctcccacgatcccaaaatggcaaaatgtgagctcatcgagttgcaggacttgactccgaatgaccgtattgagctggcaccccctagtgtccctccacccaccgtggtgcccactctggacaggtggagcagagggaaggtggtgcgcatggtgggcgagcgcgtgcgcctggaggaccccgattggctgacgtgtaaaccaggacgaggacatgactttcagccctgcagccagacacagctgagctggtgtgacctgtgtggagagttcatctggggcctgtacagacagagcctccgctgcacacactgtaactacacttgtcactaccgctgtcaacccttcattcagctggactgcagctccaacaccgacactatctgcgaacaatcaaactacagcgaggacaccatcgagacagacaccaatgtggatgagcagtctgaagtggactggaggaaacaggatctgtctgtcactgaaatacagcagaaagtgaaggaatacaatgctcaggtcaacagtaacctcttcatggttctgaatcgtgacggctcatacactggcttcatcaaggtccagtttaagctggcgcgacccgtgtctcttcctcctccccgcagcgtctcctcctcctccatctcctcctcttgtttaggatgggatggcggctgtcaggagcgaacttccttctacctgcccagagacacagtcaagcacctgcacatcagctccagcacccgtgccagagaggtcatccaggccctgctcaacaagttcactgtggtggacaatccggctaaatattccctgtatgagcgcagccagcgggacaatcaagtgtacttaaggaagttagctgatgatgaatgtccacttttcctgcgtctgtgtgctggacccaatgagaaagtcctgagtttagtgcttaaagagaatgaaaccggggaagtgaattgggatgcgttcagttttcctgaactccagaacttcctgcggattctccagcgggaggaagaagatcacgtccggcaaatcatacgccgatacactctggctcgtgataagatgaaagaggctatgaagaacttcagcaagcctggctgaatgaatctgtgtttatacctcacaaacaagagagatcgaggaggaaacaaggcttattactgtctgagtccaaagagtgtgtgaaagagcccttcgtcctactgtggacataatgagggttgaaagtgaaatgcagtgagcgagagaagagatgcgtgtgtttgaagcatgactgttgagtgtgacttcacactggaggaaatgctgcgctcgtagccgtagatccagtggagagatgtcttcctgtggagaatctatatatcagtgcagattacagagtattttcagcaccatttaaacttgtcataggaaattaaacgaggattattttaatatctgtatcaaaatgccacctgttagtgacacagtaacttgtcatattttgaagctcccatgtatatatttggatgtttgttgtcaattattctgaaaatagatacaaataaactatttttccctttaaaatga

SEQ ID NO: 2 - DNA, 420 bp, Danio rerio
atcagaacgagacgctaaatttatcagcttgctttggagtaaacagcgttgctttaaaacactccacagtcataaatcatctccagccctaaccatggtccactgagccatgccgttcatcctcccacgatcccaaaatggcaaaatgtgagctcatcgagttgcaggacttgactccgaatgaccgtattgagctggcaccccctagtgtccctccacccaccgtggtgcccactctggacaggtggagcagagggaaggtggtgcgcatggtgggcgagcgcgtgcgcctggaggaccccgattggctgacgtgtaaaccaggacgaggacatgactttcagccctgcagccagacacagctgagctggtgtgacctgtgtggagagttcatctggggcctgtacagacagagcctcc

SEQ ID NO: 3 - DNA, 420 bp, Danio rerio
attagaacgagacgttaaatttattagtttgttttggagtaaatagcgttgttttaaaatattttatagttataaattatttttagttttaattatggtttattgagttatgtcgtttatttttttacgattttaaaatggtaaaatgtgagtttatcgagttgtaggatttgatttcgaatgatcgtattgagttggtattttttagtgtttttttatttatcgtggtgtttattttggataggtggagtagagggaaggtggtgcgtatggtgggcgagcgcgtgcgtttggaggatttcgattggttgacgtgtaaattaggacgaggatatgatttttagttttgtagttagatatagttgagttggtgtgatttgtgtggagagtttatttggggtttgtatagatagagttttc

SEQ ID NO: 4 - DNA, 15 bp, Artificial sequence
  Synthetic primer/probe
cgcatggtgggcgag

SEQ ID NO: 5 - DNA, 18 bp, Artificial sequence
  Synthetic primer/probe
acacgtcagccaatcggg

SEQ ID NO: 6 - DNA, 20 bp, Artificial sequence
  Synthetic primer/probe
gacgcggaggcgcgtgcgcc

SEQ ID NO: 7 - DNA, 17 bp, Artificial sequence
  Synthetic primer/probe
tgcgtatggtgggcgag

SEQ ID NO: 8 - DNA, 26 bp, Artificial sequence
  Synthetic primer/probe
cctaatttacacgtcaaccaatcgaa

SEQ ID NO: 9 - DNA, 21 bp, Artificial sequence
  Synthetic primer/probe
gacgcggaggcgcgtgcgttt

SEQ ID NO: 10 - DNA, 21 bp, Artificial sequence
  Synthetic primer/probe
ccacggacggcgcgtgcgttt

SEQ ID NO: 11 - DNA, 171 bp, Artificial sequence
  Synthetic primer/probe
tccacgtggtgcccactctggacaggtggagcagagggaaggtggtggcatggtggggagggtggcctggaggacccgattggctgagtgtaaaccaggagaggacatgactttcagccctgcagccagacacagctgagctggtgtgacctgtgtggagagttcatctgg

SEQ ID NO: 12 - DNA, 171 bp, Artificial sequence
  Synthetic primer/probe
ccagatgaactctccacacaggtcacaccagctcagctgtgtctggctgcagggctgaaagtcatgtcctgtcctggtttacagtcagccaatggggtcctccagggcaggctgcccaccatggcaccaccttccctctgctccacctgtccagagtgggcaccaggtgga

SEQ ID NO: 13 - DNA, 224 bp, Artificial sequence
  Synthetic primer/probe
ctctgacctgagtctcctttggaactctgcaggttctatttgctttttcccagatgagctctttttctggtgtttgtctctctgactaggtgtctaagacagtgttgtgggtgtaggtactaacactggctcgtgtgacaaggccatgaggctggtgtaaagcggccttggagtgtgtattaagtaggtgcacagtaggtctgaacagactccccatcccaaga

SEQ ID NO: 14 - DNA, 224 bp, Artificial sequence
  Synthetic primer/probe
ttttgatttgagttttttttggaattttgtaggttttatttgtttttttttagatgagttttttttttggtgtttgtttttttgattaggtgtttaagatagtgttgtgggtgtaggtattaatattggtttgtgtgataaggttatgaggttggtgtaaagtggttttggagtgtgtattaagtaggtgtatagtaggtttgaatagattttttattttaaga

SEQ ID NO: 15 - DNA, 19 bp, Artificial sequence
  Synthetic primer/probe
ccatgaggctggtgtaaag

SEQ ID NO: 16 - DNA, 24 bp, Artificial sequence
  Synthetic primer/probe
ctactgtgcacctacttaatacac

SEQ ID NO: 17 - DNA, 20 bp, Artificial sequence
  Synthetic primer/probe
cgccgagggcggccttggag

SEQ ID NO: 18 - DNA, 30 bp, Artificial sequence
  Synthetic primer/probe
gtgtttgtttttttgattaggtgtttaaga

SEQ ID NO: 19 - DNA, 26 bp, Artificial sequence
  Synthetic primer/probe
ctttacaccaacctcataaccttatc

SEQ ID NO: 20 - DNA, 21 bp, Artificial sequence
  Synthetic primer/probe
gacgcggagatagtgttgtgg

SEQ ID NO: 21 - DNA, 29 bp, Artificial sequence
  Synthetic primer/probe
agccggttttccggctgagactccgcgtc

SEQ ID NO: 22 - DNA, 29 bp, Artificial sequence
  Synthetic primer/probe
agccggttttccggctgagacgtccgtgg

SEQ ID NO: 23 - DNA, 19 bp, Artificial sequence
  Synthetic primer/probe
gcgcgtccgcgcgtgcgcc

SEQ ID NO: 24 - DNA, 28 bp, Artificial sequence
  Synthetic primer/probe
agccggttttccggctgagaggacgcgc